European Patent Application EP 4 394 039 A1, published July 3, 2024. Title: L-ALANINE-PRODUCING GENETICALLY ENGINEERED STRAIN AND METHOD OF CONSTRUCTION AND USE THEREOF. Applicant: Anhui BBCA Biochemical Co., Ltd. The sequence listing filed with the application follows.

SEQUENCE LISTING (32 sequences)

SEQ ID NO: 3 - DNA, 1119 bp, Artificial Sequence
atgaaaatcggcatcccgaaagaaatcaaaaacaacgaaaaccgcgtcgcgatcacgccggcgggcgtcatgacgctggtcaaagcgggccatgacgtctatgtcgaaacggaagcgggcgcgggcagcggctttagcgacagcgaatatgaaaaagcgggcgcggtcatcgtcccgaacgcggaagacgcgtggacggcggaaatggtcctgaaagtcaaagaaccgctggcggaagaatttcgctattttcgcccgggcctgatcctgtttacgtatctgcatctggcggcggcggaagcgctgacgaaagcgctggtcgaacagaaagtcgtcggcatcgcgtatgaaacggtccagctggcgaacggcagcctgccgctgctgacgccgatgagcgaagtcgcgggccgcatgagcgtccaggtcggcgcgcagtttctggaaaaaccgcatggcggcaaaggcatcctgctgggcggcgtcccgggcgtccgccgcggcaaagtcacgatcatcggcggcggcacggcgggcacgaacgcggcgaaaatcgcggtcggcctgggcagcgacgtcacgatcctggacatcaacgcggaacgcctgcgcgaactggacgacctgtttggcgaccatgtcacgacgctgatgagcaacagctatcatatcgcggaatgcgtccgcgaaagcgacctggtcgtcggcgcggtcctgatcccgggcgcgaaagcgccgaaactggtcacggaagaaatggtccgcagcatgacgccgggcagcgtcctggtcgacatcgcgatcgaccagggcggcatctttgaaacgacggaccgcgtcacgacgcatgacgacccgacgtatgtcaaacatggcgtcgtccattatgcggtcgcgaacatgccgggcgcggtcccgcgcacgagcacgtttgcgctgacgaacgtcacgatcccgtatgcgctgcagatcgcgaacaaaggctatcgcgcggcgtgcctggacaacccggcgctgctgaaaggcatcaacacgctggacggccatatcgtctatgaagcggtcgcggcggcgcataacatgccgtatacggacgtccatagcctgctgcatggctaa

SEQ ID NO: 2 - DNA, 300 bp, Artificial Sequence
aaggtgacgcctatttcactttctagctgtttaatctgctggctgagcggaggctgagtcatgttcagccgaagagctgcttttccgaaatgcagttcttcggcaacaaccataaaataacgaagatggcgcagctccattaatcactcattcctttctgaatgcgatttcagtcgttttacatattaattgtaagacaaagaagtattggaaaacaatttccacaagatgtatatttaataatacaataattttattaaaaattcattgtaaatgaatgaaaatggaggagtgagggct

SEQ ID NO: 3 - DNA, 48 bp, Artificial Sequence
cctcgcgtcgggcgatatcggatccgaaggggaaagtcttcgatttct

SEQ ID NO: 4 - DNA, 37 bp, Artificial Sequence
agagggctttttcatgctgaagaggtcaaaaagagcc

SEQ ID NO: 5 - DNA, 38 bp, Artificial Sequence
tttgacctcttcagcatgaaaaagccctctttgaaaag

SEQ ID NO: 6 - DNA, 47 bp, Artificial Sequence
ccatggtacccgggagctcgaattccataagaccgctgatgacaagc

SEQ ID NO: 7 - DNA, 47 bp, Artificial Sequence
tccagcctcgcgtcgggcgatatcgtccccataacaacggaatcatc

SEQ ID NO: 8 - DNA, 37 bp, Artificial Sequence
aataggcgtcaccttgactcatcattcctttgccgtt

SEQ ID NO: 9 - DNA, 38 bp, Artificial Sequence
aaggaatgatgagtcaaggtgacgcctatttcactttc

SEQ ID NO: 10 - DNA, 36 bp, Artificial Sequence
tccaattcgcttcatagccctcactcctccattttc

SEQ ID NO: 11 - DNA, 39 bp, Artificial Sequence
ggaggagtgagggctatgaagcgaattggagtattgaca

SEQ ID NO: 12 - DNA, 36 bp, Artificial Sequence
cttcatggtgttcagttacaatacagtcgcatggcc

SEQ ID NO: 13 - DNA, 42 bp, Artificial Sequence
gcgactgtattgtaactgaacaccatgaagatactaacatca

SEQ ID NO: 14 - DNA, 48 bp, Artificial Sequence
actagacagatctatcgatgcatgctttcccttattcctttaaacccg

SEQ ID NO: 15 - DNA, 37 bp, Artificial Sequence
aataggcgtcaccttgctgaagaggtcaaaaagagcc

SEQ ID NO: 16 - DNA, 39 bp, Artificial Sequence
tttgacctcttcagcaaggtgacgcctatttcactttct

SEQ ID NO: 17 - DNA, 36 bp, Artificial Sequence
agagggctttttcatttagccatgcagcaggctatg

SEQ ID NO: 18 - DNA, 38 bp, Artificial Sequence
ctgctgcatggctaaatgaaaaagccctctttgaaaag

SEQ ID NO: 19 - DNA, 50 bp, Artificial Sequence
cctcgcgtcgggcgatatcggatccaaaatatgacgctgtctcaaattga

SEQ ID NO: 20 - DNA, 40 bp, Artificial Sequence
ctaattcatcaatttgacacttcctgttccttgtttcact

SEQ ID NO: 21 - DNA, 39 bp, Artificial Sequence
ggaacaggaagtgtcaaattgatgaattagcggaaaaac

SEQ ID NO: 22 - DNA, 48 bp, Artificial Sequence
ccatggtacccgggagctcgaattccggagtctctttcaaaaccgtag

SEQ ID NO: 23 - DNA, 47 bp, Artificial Sequence
cctcgcgtcgggcgatatcggatccaaaatcatgtaagcccattccg

SEQ ID NO: 24 - DNA, 37 bp, Artificial Sequence
gtgagtatgggaaaacaacgctcccttctttcttgtc

SEQ ID NO: 25 - DNA, 36 bp, Artificial Sequence
aagaagggagcgttgttttcccatactcacaggccg

SEQ ID NO: 26 - DNA, 47 bp, Artificial Sequence
ccatggtacccgggagctcgaattctaaaatgaaggtggtccgggat

SEQ ID NO: 27 - DNA, 963 bp, Bacillus coagulans
atgaagcgaattggagtattgacaagcggcggcgatgcaccggggatgaatgcggcggtccgcgcgattgcccgtaaagggatttatcacggcctggaagtttacggcattcgccaaggttataacggattgattcaaggaaacatccaaaagctcgaagcaggatctgttggcgatattctccagcggggcggcacggttttgcagtcggcaagaagcgaagaattcaaaacgccggaagggcagcaaaaagcgatcaggcagctgaaagaccatggcattgaagcgctcgttgtgatcggcggcgacggttcctaccaaggggccaaaaagttgacggaacagggctttaactgcattggtgtgccagggacaatcgataacgacatcccggggacggattttacaatcggttttgatacggcattgaacacagtgcttgatgcgattgataaaattcgcgacaccgcttcttcccacgaacgcacctttattattgaagtcatgggcagaaatgccggggatatcgcgctctggtccggcctggccggcggagccgaatcgattattattccggaagaaaaatatgacttaaaagatgtcgtggagcgtcttgaacaggggagaaaacgcggcaaacgccacagcatcatcattgtcgcggaaggcgtgatgagcggcaacgagtttgctgaacaattgaaaaaaaccggtgtgatcggcgatacccgcgtttctgttctcggccatatccagcgcggcggttctccgacggcatttgaccgcgtgcttgcaagccgcctcggcgcaagggctgttgaactgctgcttgaaggaaaagggggccgcgctgtcggcattcaaaataaccagctggttgaccacgatatccttgagattctcggaaaaccgcacgccgttaataaaaacatgtacaagctgtcgaaagaattgtcgatctaa

SEQ ID NO: 28 - DNA, 1761 bp, Bacillus coagulans
atgaaaaaaaccaaaattgtatgtacaatcggacctgccagtgaaagtgtggaaatgcttgaaagattaatggcaaacgggatggatgtttgccgcctgaacttctcgcacggcagccatgaggaacatcttgcccggattaaaaatatccgtgaagctgcaaaaaaccaaaacaaaacgatcgggcttctgctcgatacaaagggcccggaaatccgcacccatgatatgaaagacggcggattcgagctcgttgaaggcatgacaccggtcatttcaatgacagaagtgctcgggacaccggaaaaattttcggtcacatatgaagggctgattgatgatgtgcacgttggctctaaaattttacttgatgacggtttgattgaactggaagtgacggccatcgataaaaacgccggtgaaatccatacaaaagtgctgaaccgcggcgttttgaaaaacaaaaaaggtgttaacgtcccgggtgtttccgtgaaccttccgggcatcaccgaaaaagacgtgagcgatatcctgttcgggcttgaacaaggcattgacttcattgcggcttcgtttgtacgccggccgtccgacgttttggaaatccgccagctccttgaagaacacgatgctttgcatgtgaaaattttccctaaaattgaaaaccaggaaggcgtcgacaatatcgatgaaatccttgcggtatcagacggcttaatggttgcccgcggcgacctcggcgttgaaattccgaccgaagcggtgccgctcgtacaaaaagaaatgatcagaaaatgtaatacgctcggcaaaccggtgattaccgcaacgcaaatgcttgattcgatgcaacgcaacccgcgcccgacccgcgcggaagcaagcgacgtggccaacgccatttttgacggcacggatgcgatcatgctttccggcgaaacggcagccgggaaatatcctgctgaagcggttaagacgatgtacaatattgcggttcatgtggaaaaagcaattaaccatcgcgatattctgaacaagcgcagcaagagcacggaccataatatgacagacgctatctgccagtccgttgcccatacggctttaaatcttgatgtgaatgccattattgcgccgactgaaagcggctatacggcacgcatgatctccaaataccgcccggcggccccaatcattgctgtcacgagcgatccgaaagtacaacgcggcttaactgttgtgtccggcgtatacccacaattgggcacaaaggcaaacaatacggatgaaatgcttgaaattgcagtggaggaagcgttgaaatccgaaatcgtccatcacggcgaccttgtgatcattacagcaggcgtcccggttggtgggaaaggcaccaccaacctgatgaaagtgcacctgatcggtgatatattggcaaaaggccagggaatcggcagaaaatcggcattcggcccggtcatcgttgctgaaagccctgaagaagcaaacgcaaaggcaacagaaggttgtgtgctcgtcacgagaacgaccgacaaagaaatcatgccggccattgaaaaatgcgccgcgctgattacggaagaaggcggcttgacaagccatgctgcagttgttggcatcaatgtcggcattccggtcattgttggcgttgaaaaagccgtttccatttttgaagacgggcaggaagttacggtagatgcggcaaccggctcggtttacaacggccatgcgactgtattgtaa

SEQ ID NO: 29 - DNA, 1173 bp, Bacillus licheniformis
atgatgagcttaaaaccattctatagaaagacatgggccgaaatcgatttaacggctttaaaagaaaacgtccgcaatatgaagcggcacatcggcgagcatgtccgcctgatggccgtcgttaaagcgaatgcctacggacacggggatgcacaggtagcgaaggcggctcttgcagaaggggcgtccattcttgctgtggctttattggatgaagcgctttcgctgagggcgcaggggattgaagaaccgattcttgtcctcggtgcagtgccgaccgaatatgcaagcattgccgcggaaaagcgcattatcgtgactggctactccgtcggctggctgaaagacgtgctcggttttctgaatgaggccgaagctcctcttgaatatcatttgaagatcgacacgggcatgggccgccttggctgcaaaacggaagaagagatcaaagaaatgatggagatgaccgaatcgaacgataagctcaattgtacgggcgtgttcactcatttcgccacggcggacgaaaaggacaccgattatttcaacatgcagcttgaccgctttaaagagctgatcagccccctcccgcttgaccgtttgatggtgcattcgtcaaacagcgccgcgggtctgcgcttcagggaacagctatttaatgccgtccgcttcggcatcggcatgtacggtttggcgccgtcaaccgaaataaaagacgagctgccgtttcgtctgcgggaagtgttttcgcttcataccgaactcacccatgtgaaaaaaattaaaaaaggcgagagcgtcagctacggggcgacatatacagctcagcgcgacgaatggatcgggacagtccccgtcgggtatgccgacggatggctgaggcgcctggccggaacggaagtgctgatcgacggaaaacgccaaaaaatagcagggagaatctgcatggaccagttcatgatttcccttgccgaagaataccctgtcggcacaaaggttaccttgatcggaaagcaaaaagacgaatggatctcagtcgacgaaatcgcccaaaatttgcagacgatcaattatgaaattacctgtatgataagttcaagggtgccccgtatgtttttggaaaatgggagtataatggaaataaggaatccgatcttgcctgatcaatcctga

SEQ ID NO: 30 - DNA, 1182 bp, Bacillus licheniformis
atgaaaaagctttgccgtgaagtttgggtagaggtaaatcttgatgcgatcaaaaaaaatttgcgcgcgtttcggcggcatattccgaaaaagagcaaaattatggctgtcgtaaaagcgaatgcttatggtcacggatcggtggaagttgcacgccatgcacttgaacatggtgcgagtgagctcgccgttgcctcggtggaggaagcggtcgttttacgaaaagcggggattaaagcgccgatccttgtgcttggtttcaccccgctgagctgtgtgaaagaagcggcagcttggaatatatcgttatcagcttttcaagttgactggattaaagaagcgaacgagatattggaaaatgaagcagatcctaaccggctggctgttcatatcaatgtggataccggcatggggcgtttaggtgtacgaacaaaggaaaagcttttagcaatcgtggaagcgctgacggcaagtgaaaacctcgaatgggaaggaatttttacgcatttttccacagctgacgaaccggatactgagctaaccatgattcaacacgaaaagtttatcagctttcttcgctttctgaaagaacaaggctttaagctgcctacggtgcatatgaacaatacggccgcggcgatcgcttttccggaattcagcgctgatatgattcgcttaggcatcggaatgtatggattatatccttccgattatatcaggcagcttaatctcgttaagcttgtgcctgcactaagcttgaaggcgcgaatcgcttatgtgaaaaccatgttgactgaaccgcggacggttagttatggtgctacatatgttgcagagcgcggggaagtcattgccacaattccggtcggctatgctgacggctattcccgtgaactttccaaccgcggttttattcttcatcgaggaagacgagtgccggtggcgggaagagtaacaatggatatgataatggtcagtctgggagagggtgaaggtaaacaaggagaggaagtcgtgatttacggccggcaaaagggagcagagatatctgttgatgaaattgcggaaatgcttgatacgatcaactatgaagtggtatctaccataagctggcgcgtccctcgtttttatataagagacggcgagatttttaaaaagtcgaccccgctgttatacgtgtag

SEQ ID NO: 31 - DNA, 978 bp, Bacillus licheniformis
atgaaagtaatttttttttctatgcacccgtatgaagaggaatttctgggtccgattctgccgtctgactgggacgtagaaatgaccccggactttctggacgaaaccaccgtggaaaaggctaaaggtgcccaggtagtaagcctgtttgtttctgacaaagctgatggtccggtactggaagcgctgcattcttacggtgtgggcctgctggccctgcgttctgctggctatgatcacatcgatattgagaccgcaaaacgcctgggtatcaaagtagttaacgtgccagcctattctccgcacgctatcgctgaccatactctggctatcatgctggctctgattcgtcgtctgcaccgtgcccatgataaagtgcgcctgggtgattttgatctggatggtctgatgggctttgatctgaacggcaaagttgctggtgtaattggtctgggtaaaatcggtcgcctggtagctacccgcctgaaagcgtttggttgcaaagttctgggctatgatccatacattcagccggaaatcgtagaaaacgttgatctggataccctgatcactcaggctgatatcatttctattcattgtccgctgacccgtgaaaactttcatatgtttaacgaagagacttttaagcgtatgaaaccgggtgctattctggttaacaccgcgcgtggtggtctgatcgataccaaggccctgctggaggccctgaagtctggtaaactgggcggcgcagccctggatgtgtatgaatatgaacgtggcctgttttttaaaaaccaccaaaaagaaggtatcaaagacccgtatctggcccagctgctgggtctggccaacgtagtgctgaccggtcatcaggcctttctgacccgtgaggctgtaaaaaacatcgaagaaactaccgtagaaaacattctggaatggcaaaagaacccgcaggcaaagctgaaaaacgaaatctaa

SEQ ID NO: 32 - protein, 372 aa, Artificial Sequence
MKIGIPKEIKNNENRVAITPAGVMTLVKAGHDVYVETEAGAGSGFSDSEYEKAGAVIVPNAEDAWTAEMVLKVKEPLAEEFRYFRPGLILFTYLHLAAAEALTKALVEQKVVGIAYETVQLANGSLPLLTPMSEVAGRMSVQVGAQFLEKPHGGKGILLGGVPGVRRGKVTIIGGGTAGTNAAKIAVGLGSDVTILDINAERLRELDDLFGDHVTTLMSNSYHIAECVRESDLVVGAVLIPGAKAPKLVTEEMVRSMTPGSVLVDIAIDQGGIFETTDRVTTHDDPTYVKHGVVHYAVANMPGAVPRTSTFALTNVTIPYALQIANKGYRAACLDNPALLKGINTLDGHIVYEAVAAAHNMPYTDVHSLLHG